European Patent Application EP 4 414 706 A2, published August 14, 2024. Title: COLOCALIZATION-BY-LINKAGE SANDWICH ASSAYS. Applicant: Nomic Bio Inc. Application EP, filed April 3, 2019. The sequence listing filed with the application follows.

SEQUENCE LISTING (16 sequences)

SEQ ID NO: 1 - DNA, 42 bp, synthetic construct
  misc_feature 1..42: note = CLAMP Capture Oligo
  misc_feature 1: note = Biotin
  source 1..42: mol_type = other DNA
tttttttttgtggcggcggtgattggttattgagagtttatg

SEQ ID NO: 2 - DNA, 21 bp, synthetic construct
  misc_feature 1..21: note = CLAMP Spacer Oligo
  misc_feature 1: note = Biotin
  source 1..21: mol_type = other DNA
tttttttttgtggcggcggtg

SEQ ID NO: 3 - DNA, 21 bp, synthetic construct
  misc_feature 1..21: note = CLAMP Encoder Oligo
  source 1..21: mol_type = other DNA
caccgccgccacaaaaaaaaa

SEQ ID NO: 4 - DNA, 21 bp, synthetic construct
  misc_feature 1..21: note = CLAMP Encoder Oligo (FAM)
  misc_feature 21: note = FAM
  source 1..21: mol_type = other DNA
caccgccgccacaaaaaaaaa

SEQ ID NO: 5 - DNA, 21 bp, synthetic construct
  misc_feature 1..21: note = CLAMP Encoder Oligo (Cy3)
  misc_feature 21: note = Cy3
  source 1..21: mol_type = other DNA
caccgccgccacaaaaaaaaa

SEQ ID NO: 6 - DNA, 81 bp, synthetic construct
  misc_feature 1..81: note = CLAMP Hook Oligo
  misc_feature 1: note = Thiol
  source 1..81: mol_type = other DNA
ttttttacttttcaaccaccactcaaccatattcaactcattcgccataaactcattcgccataaactctcaataaccaat

SEQ ID NO: 7 - DNA, 81 bp, synthetic construct; identical to SEQ ID NO: 6
  misc_feature 1..81: note = CLAMP Hook Oligo
  misc_feature 1: note = Cy5
  source 1..81: mol_type = other DNA

SEQ ID NO: 8 - DNA, 30 bp, synthetic construct
  misc_feature 1..30: note = CLAMP Displacer Oligo
  misc_feature 30: note = Cy5
  source 1..30: mol_type = other DNA
attggttattgagagtttatggcgaatgag

SEQ ID NO: 9 - DNA, 30 bp, synthetic construct; identical to SEQ ID NO: 8
  misc_feature 1..30: note = CLAMP Displacer Oligo
  source 1..30: mol_type = other DNA

SEQ ID NO: 10 - DNA, 30 bp, synthetic construct
  misc_feature 1..30: note = CLAMP Labeler Oligo
  source 1..30: mol_type = other DNA
gttgagtggtggttgattggttgggattga

SEQ ID NO: 11 - DNA, 45 bp, synthetic construct
  misc_feature 1..45: note = HOP-MPs Capture Oligo (2)
  misc_feature 1: note = Biotin
  source 1..45: mol_type = other DNA
tttttttttgtggcggcggtggttgagtggtggttggtgttgatt

SEQ ID NO: 12 - DNA, 45 bp, synthetic construct
  misc_feature 1..45: note = HOP-MPs Displacer Oligo (2)
  source 1..45: mol_type = other DNA
ctcgtcataatgtaaaccgggaatcaacaccaaccaccactcaac

SEQ ID NO: 13 - DNA, 30 bp, synthetic construct; identical to SEQ ID NO: 8
  misc_feature 1..30: note = DO
  source 1..30: mol_type = other DNA

SEQ ID NO: 14 - DNA, 42 bp, synthetic construct; identical to SEQ ID NO: 1
  misc_feature 1..42: note = CO
  source 1..42: mol_type = other DNA

SEQ ID NO: 15 - DNA, 21 bp, synthetic construct
  misc_feature 1..21: note = LO
  source 1..21: mol_type = other DNA
caccgccgccacaaaaaaaaa

SEQ ID NO: 16 - DNA, 81 bp, synthetic construct; identical to SEQ ID NO: 6
  misc_feature 1..81: note = HO
  source 1..81: mol_type = other DNA